European Patent Specification EP 3 548 516 B1, published May 21, 2025. Title: A novel CD33-, CD16- and CD123-specific single chain triplebody. Applicant: Friedrich-Alexander-Universität Erlangen-Nürnberg Westend-Innovation UG. The sequence listing filed with the application follows.

SEQUENCE LISTING (8 sequences)

SEQ ID NO: 1 - protein, 793 aa, Artificial Sequence
  SPM-2 with HIS tag (without leader)
EVQLVESGGGLIQPGGSLRLSCAASGFPLTSYGVSWVRQPPGKGLEWLGVIWGDGSTNYHSALISRFTISRDNSKNTLYLQMNSLRAEDTAVYYCARDTYYPYYAMDYWGQGTTVTVSSGGGGSGGGGSGGGGSDIQMTQSPSSLSASVGDRVTITCKASQDVSTAVAWYQQKPGKAPKLLIYSASYRYTGVPSRFSGSGSGTDFTLTISSLQPEDFATYYCQQHYSTPLTFGQGTKLEIKRGGGGSGGGGSGGGGSGGGGSDIVLTQSPSSLSASVGDRVTITCKASQSVDFDGDSFMNWYQQKPGKAPKLLIYTTSNLESGVPSRFSASGSGTDFTLTISSLQPEDFATYYCQQSNEDPYTFGCGTKVEIKRGGGGSGGGGSGGGGSGGGGSEVQLVESGGGDVQPGGSLRLSCAFSGFSLRTSGMGVGWIRQAPGKCLEWVAHIWWDDDKRYNPSVKGRFTISKDTSSNTVYLQMNSLRAEDTAVYYCAQINPAWFAYWGQGTLVTVSSGGGGSGGGGSGGGGSGGGGSEVQLVESGGGLVQPGGSLRLSCAASGFTFTDYYMSWVRQAPGKCLEWLALIRSKADGYTTEYSASVKGRFTISRDDSKNSLYLQMNSLKTEDTAVYYCARDAAYYSYYSPEGAMDYWGQGTSVTVSSGGGGSGGGGSGGGGSDIQMTQSPSSLSASVGDRVTITCKASQNVDSAVAWYQQKPGKAPKALIYSASYRYSGVPSRFSGSGSGTDFTLTISSLQPEDFATYYCQQYYSTPWTFGCGTKVEIKRGGGGSHHHHHH

SEQ ID NO: 2 - DNA, 2382 bp, Artificial Sequence
  source 1..2382: /mol_type="unassigned DNA" /note="SPM-2 with HIS tag (without leader)" /organism="Artificial Sequence"
gaagtccaactcgttgagagcggcggagggcttattcagcctggggggtcattgcgcctctcatgtgccgcctctggtttccctctgacgagctacggcgtgtcctgggtgaggcagcctccaggaaaaggtcttgaatggttgggcgtgatctggggcgatggcagcactaactatcactccgcactgataagtagattcaccatttcccgggacaattccaagaacacgctctatcttcagatgaattccctgagagccgaggacacagcagtttactattgtgctcgggatacctactatccctactacgccatggattactggggccaagggacaactgttaccgtgagctccggcggtggaggaagtggtggaggtggcagtggcggcggtgggtccgacattcaaatgactcagagcccttctagcctctctgccagcgtgggcgaccgggtgaccatcacatgcaaggccagtcaggatgtgtccaccgccgtggcttggtatcagcaaaagcctggcaaggctcccaagctgctcatctactctgccagttatcgatataccggggttccctcacgtttcagcggctctgggtcagggactgactttactctgaccatttctagcctccaaccagaggattttgcaacttactattgtcagcagcactactctaccccactcacatttggccagggaaccaaattggagatcaagcggggcggtggtgggtccggcggcggaggcagtggcgggggaggtagcggtggcggcgggagtgatatagtcttgacccagtctccatcctccctgtccgcttcagtgggcgacagagtcacaatcacgtgcaaggccagccagtctgtcgactttgacggcgactcctttatgaattggtaccaacagaagccagggaaagctcccaagttgctgatctataccacttccaatctggaaagcggtgttccctcacgcttctcagcatcaggaagcgggacagactttacgctgaccattagctcactgcagccagaggatttcgctacatactactgccagcaatcaaacgaggatccttatacctttggctgcggaacaaaggtcgaaatcaagagaggcggaggtgggtcaggtggaggcggctctggcggaggaggtagcggaggaggcggatccgaggttcagctggtggaatccggtggcggagatgtgcagcccggaggatctctgaggctcagttgtgctttctccggcttcagtctgcgtacttcaggcatgggcgtggggtggattaggcaggcacctggtaagtgccttgagtgggtcgcccacatttggtgggatgacgacaaacggtacaatccctcagtcaagggtaggtttaccatttccaaggacacatccagcaacacagtatatctgcagatgaacagcttgagagccgaggatacagctgtctactactgcgctcagatcaaccccgcttggttcgcctattggggccaggggaccctggtgacagtgagttctggtggaggtggctcaggggggggcggttctggcggtggggggtccggggggggtggtagtgaagtccagctggtggagagtggaggagggctggtgcaacccggagggtcacttaggctgagttgcgctgcatctggcttcacattcactgactactacatgtcctgggtgcgccaggcacccggtaagtgcctggaatggcttgctctgattcgttctaaagccgatggatacactaccgaatatagtgcaagcgtcaaaggaaggttcacaatctcccgagatgactccaagaatagtctgtatctgcaaatgaactccctcaaaacagaggacaccgctgtatattactgtgcccgcgacgccgcttactacagttattactctccagaaggagccatggattattggggtcaggggacctccgttaccgtatctagtggcggaggcggttctggaggaggtggatccgggggaggcggcagcgacatccagatgacacagtcccctagctccctgtctgcatccgtgggagatcgagtgactatcacttgcaaagcaagtcagaacgtggatagcgccgttgcatggtatcagcagaagcccggaaaggccccaaaagccttgatctactccgcctcctaccggtattctggggtaccatcacgcttctctgggtctggcagcggaaccgactttaccctgactataagcagcctgcagcccgaggactttgctacctattactgtcagcagtattacagcactccttggacttttggctgtgggacgaaagtggagatcaaacgagggggcggtggctctcaccatcatcaccatcattga

SEQ ID NO: 3 - protein, 782 aa, Artificial Sequence
  SPM-2 without HIS tag (without leader)
EVQLVESGGGLIQPGGSLRLSCAASGFPLTSYGVSWVRQPPGKGLEWLGVIWGDGSTNYHSALISRFTISRDNSKNTLYLQMNSLRAEDTAVYYCARDTYYPYYAMDYWGQGTTVTVSSGGGGSGGGGSGGGGSDIQMTQSPSSLSASVGDRVTITCKASQDVSTAVAWYQQKPGKAPKLLIYSASYRYTGVPSRFSGSGSGTDFTLTISSLQPEDFATYYCQQHYSTPLTFGQGTKLEIKRGGGGSGGGGSGGGGSGGGGSDIVLTQSPSSLSASVGDRVTITCKASQSVDFDGDSFMNWYQQKPGKAPKLLIYTTSNLESGVPSRFSASGSGTDFTLTISSLQPEDFATYYCQQSNEDPYTFGCGTKVEIKRGGGGSGGGGSGGGGSGGGGSEVQLVESGGGDVQPGGSLRLSCAFSGFSLRTSGMGVGWIRQAPGKCLEWVAHIWWDDDKRYNPSVKGRFTISKDTSSNTVYLQMNSLRAEDTAVYYCAQINPAWFAYWGQGTLVTVSSGGGGSGGGGSGGGGSGGGGSEVQLVESGGGLVQPGGSLRLSCAASGFTFTDYYMSWVRQAPGKCLEWLALIRSKADGYTTEYSASVKGRFTISRDDSKNSLYLQMNSLKTEDTAVYYCARDAAYYSYYSPEGAMDYWGQGTSVTVSSGGGGSGGGGSGGGGSDIQMTQSPSSLSASVGDRVTITCKASQNVDSAVAWYQQKPGKAPKALIYSASYRYSGVPSRFSGSGSGTDFTLTISSLQPEDFATYYCQQYYSTPWTFGCGTKVEIKR

SEQ ID NO: 4 - DNA, 2349 bp, Artificial Sequence
  source 1..2349: /mol_type="unassigned DNA" /note="SPM-2 without HIS tag (without leader)" /organism="Artificial Sequence"
gaagtccaactcgttgagagcggcggagggcttattcagcctggggggtcattgcgcctctcatgtgccgcctctggtttccctctgacgagctacggcgtgtcctgggtgaggcagcctccaggaaaaggtcttgaatggttgggcgtgatctggggcgatggcagcactaactatcactccgcactgataagtagattcaccatttcccgggacaattccaagaacacgctctatcttcagatgaattccctgagagccgaggacacagcagtttactattgtgctcgggatacctactatccctactacgccatggattactggggccaagggacaactgttaccgtgagctccggcggtggaggaagtggtggaggtggcagtggcggcggtgggtccgacattcaaatgactcagagcccttctagcctctctgccagcgtgggcgaccgggtgaccatcacatgcaaggccagtcaggatgtgtccaccgccgtggcttggtatcagcaaaagcctggcaaggctcccaagctgctcatctactctgccagttatcgatataccggggttccctcacgtttcagcggctctgggtcagggactgactttactctgaccatttctagcctccaaccagaggattttgcaacttactattgtcagcagcactactctaccccactcacatttggccagggaaccaaattggagatcaagcggggcggtggtgggtccggcggcggaggcagtggcgggggaggtagcggtggcggcgggagtgatatagtcttgacccagtctccatcctccctgtccgcttcagtgggcgacagagtcacaatcacgtgcaaggccagccagtctgtcgactttgacggcgactcctttatgaattggtaccaacagaagccagggaaagctcccaagttgctgatctataccacttccaatctggaaagcggtgttccctcacgcttctcagcatcaggaagcgggacagactttacgctgaccattagctcactgcagccagaggatttcgctacatactactgccagcaatcaaacgaggatccttatacctttggctgcggaacaaaggtcgaaatcaagagaggcggaggtgggtcaggtggaggcggctctggcggaggaggtagcggaggaggcggatccgaggttcagctggtggaatccggtggcggagatgtgcagcccggaggatctctgaggctcagttgtgctttctccggcttcagtctgcgtacttcaggcatgggcgtggggtggattaggcaggcacctggtaagtgccttgagtgggtcgcccacatttggtgggatgacgacaaacggtacaatccctcagtcaagggtaggtttaccatttccaaggacacatccagcaacacagtatatctgcagatgaacagcttgagagccgaggatacagctgtctactactgcgctcagatcaaccccgcttggttcgcctattggggccaggggaccctggtgacagtgagttctggtggaggtggctcaggggggggcggttctggcggtggggggtccggggggggtggtagtgaagtccagctggtggagagtggaggagggctggtgcaacccggagggtcacttaggctgagttgcgctgcatctggcttcacattcactgactactacatgtcctgggtgcgccaggcacccggtaagtgcctggaatggcttgctctgattcgttctaaagccgatggatacactaccgaatatagtgcaagcgtcaaaggaaggttcacaatctcccgagatgactccaagaatagtctgtatctgcaaatgaactccctcaaaacagaggacaccgctgtatattactgtgcccgcgacgccgcttactacagttattactctccagaaggagccatggattattggggtcaggggacctccgttaccgtatctagtggcggaggcggttctggaggaggtggatccgggggaggcggcagcgacatccagatgacacagtcccctagctccctgtctgcatccgtgggagatcgagtgactatcacttgcaaagcaagtcagaacgtggatagcgccgttgcatggtatcagcagaagcccggaaaggccccaaaagccttgatctactccgcctcctaccggtattctggggtaccatcacgcttctctgggtctggcagcggaaccgactttaccctgactataagcagcctgcagcccgaggactttgctacctattactgtcagcagtattacagcactccttggacttttggctgtgggacgaaagtggagatcaaacgatga

SEQ ID NO: 5 - protein, 813 aa, Artificial Sequence
  SPM-2 with leader sequence and HIS tag
METDTLLLWVLLLWVPGSTGEVQLVESGGGLIQPGGSLRLSCAASGFPLTSYGVSWVRQPPGKGLEWLGVIWGDGSTNYHSALISRFTISRDNSKNTLYLQMNSLRAEDTAVYYCARDTYYPYYAMDYWGQGTTVTVSSGGGGSGGGGSGGGGSDIQMTQSPSSLSASVGDRVTITCKASQDVSTAVAWYQQKPGKAPKLLIYSASYRYTGVPSRFSGSGSGTDFTLTISSLQPEDFATYYCQQHYSTPLTFGQGTKLEIKRGGGGSGGGGSGGGGSGGGGSDIVLTQSPSSLSASVGDRVTITCKASQSVDFDGDSFMNWYQQKPGKAPKLLIYTTSNLESGVPSRFSASGSGTDFTLTISSLQPEDFATYYCQQSNEDPYTFGCGTKVEIKRGGGGSGGGGSGGGGSGGGGSEVQLVESGGGDVQPGGSLRLSCAFSGFSLRTSGMGVGWIRQAPGKCLEWVAHIWWDDDKRYNPSVKGRFTISKDTSSNTVYLQMNSLRAEDTAVYYCAQINPAWFAYWGQGTLVTVSSGGGGSGGGGSGGGGSGGGGSEVQLVESGGGLVQPGGSLRLSCAASGFTFTDYYMSWVRQAPGKCLEWLALIRSKADGYTTEYSASVKGRFTISRDDSKNSLYLQMNSLKTEDTAVYYCARDAAYYSYYSPEGAMDYWGQGTSVTVSSGGGGSGGGGSGGGGSDIQMTQSPSSLSASVGDRVTITCKASQNVDSAVAWYQQKPGKAPKALIYSASYRYSGVPSRFSGSGSGTDFTLTISSLQPEDFATYYCQQYYSTPWTFGCGTKVEIKRGGGGSHHHHHH

SEQ ID NO: 6 - DNA, 2442 bp, Artificial Sequence
  source 1..2442: /mol_type="unassigned DNA" /note="SPM-2 with leader sequence and HIS tag" /organism="Artificial Sequence"
atggagactgatacattgctgctctgggtactgcttctgtgggtccctggttctaccggcgaagtccaactcgttgagagcggcggagggcttattcagcctggggggtcattgcgcctctcatgtgccgcctctggtttccctctgacgagctacggcgtgtcctgggtgaggcagcctccaggaaaaggtcttgaatggttgggcgtgatctggggcgatggcagcactaactatcactccgcactgataagtagattcaccatttcccgggacaattccaagaacacgctctatcttcagatgaattccctgagagccgaggacacagcagtttactattgtgctcgggatacctactatccctactacgccatggattactggggccaagggacaactgttaccgtgagctccggcggtggaggaagtggtggaggtggcagtggcggcggtgggtccgacattcaaatgactcagagcccttctagcctctctgccagcgtgggcgaccgggtgaccatcacatgcaaggccagtcaggatgtgtccaccgccgtggcttggtatcagcaaaagcctggcaaggctcccaagctgctcatctactctgccagttatcgatataccggggttccctcacgtttcagcggctctgggtcagggactgactttactctgaccatttctagcctccaaccagaggattttgcaacttactattgtcagcagcactactctaccccactcacatttggccagggaaccaaattggagatcaagcggggcggtggtgggtccggcggcggaggcagtggcgggggaggtagcggtggcggcgggagtgatatagtcttgacccagtctccatcctccctgtccgcttcagtgggcgacagagtcacaatcacgtgcaaggccagccagtctgtcgactttgacggcgactcctttatgaattggtaccaacagaagccagggaaagctcccaagttgctgatctataccacttccaatctggaaagcggtgttccctcacgcttctcagcatcaggaagcgggacagactttacgctgaccattagctcactgcagccagaggatttcgctacatactactgccagcaatcaaacgaggatccttatacctttggctgcggaacaaaggtcgaaatcaagagaggcggaggtgggtcaggtggaggcggctctggcggaggaggtagcggaggaggcggatccgaggttcagctggtggaatccggtggcggagatgtgcagcccggaggatctctgaggctcagttgtgctttctccggcttcagtctgcgtacttcaggcatgggcgtggggtggattaggcaggcacctggtaagtgccttgagtgggtcgcccacatttggtgggatgacgacaaacggtacaatccctcagtcaagggtaggtttaccatttccaaggacacatccagcaacacagtatatctgcagatgaacagcttgagagccgaggatacagctgtctactactgcgctcagatcaaccccgcttggttcgcctattggggccaggggaccctggtgacagtgagttctggtggaggtggctcaggggggggcggttctggcggtggggggtccggggggggtggtagtgaagtccagctggtggagagtggaggagggctggtgcaacccggagggtcacttaggctgagttgcgctgcatctggcttcacattcactgactactacatgtcctgggtgcgccaggcacccggtaagtgcctggaatggcttgctctgattcgttctaaagccgatggatacactaccgaatatagtgcaagcgtcaaaggaaggttcacaatctcccgagatgactccaagaatagtctgtatctgcaaatgaactccctcaaaacagaggacaccgctgtatattactgtgcccgcgacgccgcttactacagttattactctccagaaggagccatggattattggggtcaggggacctccgttaccgtatctagtggcggaggcggttctggaggaggtggatccgggggaggcggcagcgacatccagatgacacagtcccctagctccctgtctgcatccgtgggagatcgagtgactatcacttgcaaagcaagtcagaacgtggatagcgccgttgcatggtatcagcagaagcccggaaaggccccaaaagccttgatctactccgcctcctaccggtattctggggtaccatcacgcttctctgggtctggcagcggaaccgactttaccctgactataagcagcctgcagcccgaggactttgctacctattactgtcagcagtattacagcactccttggacttttggctgtgggacgaaagtggagatcaaacgagggggcggtggctctcaccatcatcaccatcattga

SEQ ID NO: 7 - protein, 802 aa, Artificial Sequence
  SPM-2 with leader sequence and without HIS tag
METDTLLLWVLLLWVPGSTGEVQLVESGGGLIQPGGSLRLSCAASGFPLTSYGVSWVRQPPGKGLEWLGVIWGDGSTNYHSALISRFTISRDNSKNTLYLQMNSLRAEDTAVYYCARDTYYPYYAMDYWGQGTTVTVSSGGGGSGGGGSGGGGSDIQMTQSPSSLSASVGDRVTITCKASQDVSTAVAWYQQKPGKAPKLLIYSASYRYTGVPSRFSGSGSGTDFTLTISSLQPEDFATYYCQQHYSTPLTFGQGTKLEIKRGGGGSGGGGSGGGGSGGGGSDIVLTQSPSSLSASVGDRVTITCKASQSVDFDGDSFMNWYQQKPGKAPKLLIYTTSNLESGVPSRFSASGSGTDFTLTISSLQPEDFATYYCQQSNEDPYTFGCGTKVEIKRGGGGSGGGGSGGGGSGGGGSEVQLVESGGGDVQPGGSLRLSCAFSGFSLRTSGMGVGWIRQAPGKCLEWVAHIWWDDDKRYNPSVKGRFTISKDTSSNTVYLQMNSLRAEDTAVYYCAQINPAWFAYWGQGTLVTVSSGGGGSGGGGSGGGGSGGGGSEVQLVESGGGLVQPGGSLRLSCAASGFTFTDYYMSWVRQAPGKCLEWLALIRSKADGYTTEYSASVKGRFTISRDDSKNSLYLQMNSLKTEDTAVYYCARDAAYYSYYSPEGAMDYWGQGTSVTVSSGGGGSGGGGSGGGGSDIQMTQSPSSLSASVGDRVTITCKASQNVDSAVAWYQQKPGKAPKALIYSASYRYSGVPSRFSGSGSGTDFTLTISSLQPEDFATYYCQQYYSTPWTFGCGTKVEIKR

SEQ ID NO: 8 - DNA, 2409 bp, Artificial Sequence
  source 1..2409: /mol_type="unassigned DNA" /note="SPM-2 with leader sequence and without HIS tag" /organism="Artificial Sequence"
atggagactgatacattgctgctctgggtactgcttctgtgggtccctggttctaccggcgaagtccaactcgttgagagcggcggagggcttattcagcctggggggtcattgcgcctctcatgtgccgcctctggtttccctctgacgagctacggcgtgtcctgggtgaggcagcctccaggaaaaggtcttgaatggttgggcgtgatctggggcgatggcagcactaactatcactccgcactgataagtagattcaccatttcccgggacaattccaagaacacgctctatcttcagatgaattccctgagagccgaggacacagcagtttactattgtgctcgggatacctactatccctactacgccatggattactggggccaagggacaactgttaccgtgagctccggcggtggaggaagtggtggaggtggcagtggcggcggtgggtccgacattcaaatgactcagagcccttctagcctctctgccagcgtgggcgaccgggtgaccatcacatgcaaggccagtcaggatgtgtccaccgccgtggcttggtatcagcaaaagcctggcaaggctcccaagctgctcatctactctgccagttatcgatataccggggttccctcacgtttcagcggctctgggtcagggactgactttactctgaccatttctagcctccaaccagaggattttgcaacttactattgtcagcagcactactctaccccactcacatttggccagggaaccaaattggagatcaagcggggcggtggtgggtccggcggcggaggcagtggcgggggaggtagcggtggcggcgggagtgatatagtcttgacccagtctccatcctccctgtccgcttcagtgggcgacagagtcacaatcacgtgcaaggccagccagtctgtcgactttgacggcgactcctttatgaattggtaccaacagaagccagggaaagctcccaagttgctgatctataccacttccaatctggaaagcggtgttccctcacgcttctcagcatcaggaagcgggacagactttacgctgaccattagctcactgcagccagaggatttcgctacatactactgccagcaatcaaacgaggatccttatacctttggctgcggaacaaaggtcgaaatcaagagaggcggaggtgggtcaggtggaggcggctctggcggaggaggtagcggaggaggcggatccgaggttcagctggtggaatccggtggcggagatgtgcagcccggaggatctctgaggctcagttgtgctttctccggcttcagtctgcgtacttcaggcatgggcgtggggtggattaggcaggcacctggtaagtgccttgagtgggtcgcccacatttggtgggatgacgacaaacggtacaatccctcagtcaagggtaggtttaccatttccaaggacacatccagcaacacagtatatctgcagatgaacagcttgagagccgaggatacagctgtctactactgcgctcagatcaaccccgcttggttcgcctattggggccaggggaccctggtgacagtgagttctggtggaggtggctcaggggggggcggttctggcggtggggggtccggggggggtggtagtgaagtccagctggtggagagtggaggagggctggtgcaacccggagggtcacttaggctgagttgcgctgcatctggcttcacattcactgactactacatgtcctgggtgcgccaggcacccggtaagtgcctggaatggcttgctctgattcgttctaaagccgatggatacactaccgaatatagtgcaagcgtcaaaggaaggttcacaatctcccgagatgactccaagaatagtctgtatctgcaaatgaactccctcaaaacagaggacaccgctgtatattactgtgcccgcgacgccgcttactacagttattactctccagaaggagccatggattattggggtcaggggacctccgttaccgtatctagtggcggaggcggttctggaggaggtggatccgggggaggcggcagcgacatccagatgacacagtcccctagctccctgtctgcatccgtgggagatcgagtgactatcacttgcaaagcaagtcagaacgtggatagcgccgttgcatggtatcagcagaagcccggaaaggccccaaaagccttgatctactccgcctcctaccggtattctggggtaccatcacgcttctctgggtctggcagcggaaccgactttaccctgactataagcagcctgcagcccgaggactttgctacctattactgtcagcagtattacagcactccttggacttttggctgtgggacgaaagtggagatcaaacgatga